European Patent Application EP 4 467 573 A1, published November 27, 2024. Title: 一种双特异性结合分子. Applicant: 苏州生物医药转化工程中心. Application CN, filed October 15, 2022. The sequence listing filed with the application follows.

SEQUENCE LISTING (26 sequences)

SEQ ID NO: 1 - protein, 447 aa, synthetic construct
EVQLVESGGGLVQPGGSLRLSCAASGFFITNNYWGWVRQAPGKGLEWVGYISYSGSTSYNPSLKSRFTISRDTSKNTFYLQMNSLRAEDTAVYYCARTGSSGYFDFWGQGTLVTVSSASTKGPSVFPLAPSSKSTSGGTAALGCLVKDYFPEPVTVSWNSGALTSGVHTFPAVLQSSGLYSLSSVVTVPSSSLGTQTYICNVNHKPSNTKVDKKVEPKSCDKTHTCPPCPAPELLGGPSVFLFPPKPKDTLMISRTPEVTCVVVDVSHEDPEVKFNWYVDGVEVHNAKTKPREEQYASTYRVVSVLTVLHQDWLNGKEYKCKVSNKALPAPIEKTISKAKGQPREPQVYTLPPSREEMTKNQVSLTCLVKGFYPSDIAVEWESNGQPENNYKTTPPVLDSDGSFFLYSKLTVDKSRWQQGNVFSCSVMHEALHNHYTQKSLSLSPGK

SEQ ID NO: 2 - protein, 214 aa, synthetic construct
DIQMTQSPSSLSASVGDRVTITCRASESVDDLLHWYQQKPGKAPKLLIKYASQSISGVPSRFSGSGSGTDFTLTISSLQPEDFATYYCQQGNSLPNTFGQGTKVEIKRTVAAPSVFIFPPSDEQLKSGTASVVCLLNNFYPREAKVQWKVDNALQSGNSQESVTEQDSKDSTYSLSSTLTLSKADYEKHKVYACEVTHQGLSSPVTKSFNRGEC

SEQ ID NO: 3 - protein, 293 aa, synthetic construct
DIQMTQSPSSLSASVGDRVTITCRASESGGSGAKLAALKAKLAALKGGGGSAAAISCVGSPECPPKCRAQGCKNGKCMNRKCKCYYCGGGGSELAALEAELAALEAGGSGLLHWYQQKPGKAPKLLIKYASQSISGVPSRFSGSGSGTDFTLTISSLQPEDFATYYCQQGNSLPNTFGQGTKVEIKRTVAAPSVFIFPPSDEQLKSGTASVVCLLNNFYPREAKVQWKVDNALQSGNSQESVTEQDSKDSTYSLSSTLTLSKADYEKHKVYACEVTHQGLSSPVTKSFNRGEC

SEQ ID NO: 4 - protein, 293 aa, synthetic construct
DIQMTQSPSSLSASVGDRVTITCRASESVDDLLHWYQQKPGKAPKLLIKYASQSISGGSGAKLAALKAKLAALKGGGGSAAAISCVGSPECPPKCRAQGCKNGKCMNRKCKCYYCGGGGSELAALEAELAALEAGGSGSRFSGSGSGTDFTLTISSLQPEDFATYYCQQGNSLPNTFGQGTKVEIKRTVAAPSVFIFPPSDEQLKSGTASVVCLLNNFYPREAKVQWKVDNALQSGNSQESVTEQDSKDSTYSLSSTLTLSKADYEKHKVYACEVTHQGLSSPVTKSFNRGEC

SEQ ID NO: 5 - protein, 292 aa, synthetic construct
DIQMTQSPSSLSASVGDRVTITCRASESVDDLLHWYQQKPGKAPKLLIKYASQSISGVPSRFSGSGSGTDFTLTISSLQPEDFATYYCQQGGGSGAKLAALKAKLAALKGGGGSAAAISCVGSPECPPKCRAQGCKNGKCMNRKCKCYYCGGGGSELAALEAELAALEAGGSGNTFGQGTKVEIKRTVAAPSVFIFPPSDEQLKSGTASVVCLLNNFYPREAKVQWKVDNALQSGNSQESVTEQDSKDSTYSLSSTLTLSKADYEKHKVYACEVTHQGLSSPVTKSFNRGEC

SEQ ID NO: 6 - protein, 523 aa, synthetic construct
EVQLVESGGGLVQPGGSLRLSCAASGGGSGAKLAALKAKLAALKGGGGSAAAISCVGSPECPPKCRAQGCKNGKCMNRKCKCYYCGGGGSELAALEAELAALEAGGSGYWGWVRQAPGKGLEWVGYISYSGSTSYNPSLKSRFTISRDTSKNTFYLQMNSLRAEDTAVYYCARTGSSGYFDFWGQGTLVTVSSASTKGPSVFPLAPSSKSTSGGTAALGCLVKDYFPEPVTVSWNSGALTSGVHTFPAVLQSSGLYSLSSVVTVPSSSLGTQTYICNVNHKPSNTKVDKKVEPKSCDKTHTCPPCPAPELLGGPSVFLFPPKPKDTLMISRTPEVTCVVVDVSHEDPEVKFNWYVDGVEVHNAKTKPREEQYASTYRVVSVLTVLHQDWLNGKEYKCKVSNKALPAPIEKTISKAKGQPREPQVYTLPPSREEMTKNQVSLTCLVKGFYPSDIAVEWESNGQPENNYKTTPPVLDSDGSFFLYSKLTVDKSRWQQGNVFSCSVMHEALHNHYTQKSLSLSPGK

SEQ ID NO: 7 - protein, 525 aa, synthetic construct
EVQLVESGGGLVQPGGSLRLSCAASGFFITNNYWGWVRQAPGKGLEWVGYISYSGSTSYNGGSGAKLAALKAKLAALKGGGGSAAAISCVGSPECPPKCRAQGCKNGKCMNRKCKCYYCGGGGSELAALEAELAALEAGGSGSRFTISRDTSKNTFYLQMNSLRAEDTAVYYCARTGSSGYFDFWGQGTLVTVSSASTKGPSVFPLAPSSKSTSGGTAALGCLVKDYFPEPVTVSWNSGALTSGVHTFPAVLQSSGLYSLSSVVTVPSSSLGTQTYICNVNHKPSNTKVDKKVEPKSCDKTHTCPPCPAPELLGGPSVFLFPPKPKDTLMISRTPEVTCVVVDVSHEDPEVKFNWYVDGVEVHNAKTKPREEQYASTYRVVSVLTVLHQDWLNGKEYKCKVSNKALPAPIEKTISKAKGQPREPQVYTLPPSREEMTKNQVSLTCLVKGFYPSDIAVEWESNGQPENNYKTTPPVLDSDGSFFLYSKLTVDKSRWQQGNVFSCSVMHEALHNHYTQKSLSLSPGK

SEQ ID NO: 8 - protein, 525 aa, synthetic construct
EVQLVESGGGLVQPGGSLRLSCAASGFFITNNYWGWVRQAPGKGLEWVGYISYSGSTSYNPSLKSRFTISRDTSKNTFYLQMNSLRAEDTAVYYCARGGSGAKLAALKAKLAALKGGGGSAAAISCVGSPECPPKCRAQGCKNGKCMNRKCKCYYCGGGGSELAALEAELAALEAGGSGGYFDFWGQGTLVTVSSASTKGPSVFPLAPSSKSTSGGTAALGCLVKDYFPEPVTVSWNSGALTSGVHTFPAVLQSSGLYSLSSVVTVPSSSLGTQTYICNVNHKPSNTKVDKKVEPKSCDKTHTCPPCPAPELLGGPSVFLFPPKPKDTLMISRTPEVTCVVVDVSHEDPEVKFNWYVDGVEVHNAKTKPREEQYASTYRVVSVLTVLHQDWLNGKEYKCKVSNKALPAPIEKTISKAKGQPREPQVYTLPPSREEMTKNQVSLTCLVKGFYPSDIAVEWESNGQPENNYKTTPPVLDSDGSFFLYSKLTVDKSRWQQGNVFSCSVMHEALHNHYTQKSLSLSPGK

SEQ ID NO: 9 - protein, 36 aa, synthetic construct
AAAISCVGSPECPPKCRAQGCKNGKCMNRKCKCYYC

SEQ ID NO: 10 - protein, 6 aa, synthetic construct
ESVDDL

SEQ ID NO: 11 - protein, 5 aa, synthetic construct
KYASQ

SEQ ID NO: 12 - protein, 9 aa, synthetic construct
QQGNSLPNT

SEQ ID NO: 13 - protein, 6 aa, synthetic construct
FFITNN

SEQ ID NO: 14 - protein, 7 aa, synthetic construct
ISYSGST

SEQ ID NO: 15 - protein, 10 aa, synthetic construct
ARTGSSGYFD

SEQ ID NO: 16 - protein, 23 aa, synthetic construct
GGSGAKLAALKAKLAALKGGGGS

SEQ ID NO: 17 - protein, 23 aa, synthetic construct
GGGGSELAALEAELAALEAGGSG

SEQ ID NO: 18 - DNA, 1341 bp, synthetic construct
  source 1..1341: mol_type = other DNA
gaggtgcagctggtggagagcggcggcggcctggtgcagcccggcggcagcctgcgcctgagctgcgccgccagcggcttcttcatcaccaacaactactggggctgggtgcgccaggcccccggcaagggcctggagtgggtgggctacatcagctacagcggcagcaccagctacaaccccagcctgaagagccgcttcaccatcagccgcgacaccagcaagaacaccttctacctgcagatgaacagcctgcgcgccgaggacaccgccgtgtactactgcgcccgcaccggcagcagcggctacttcgacttctggggccagggcaccctggtgaccgtgagcagcgcctccaccaagggcccatcggtcttccccctggcaccctcctccaagagcacctctgggggcacagcggccctgggctgcctggtcaaggactacttccccgaaccggtgacggtgtcgtggaactcaggcgccctgaccagcggcgtgcacaccttcccggctgtcctacagtcctcaggactctactccctcagcagcgtggtgactgtgccctctagcagcttgggcacccagacctacatctgcaacgtgaatcacaagcccagcaacaccaaggtggacaagaaagttgaacccaaatcttgcgacaaaactcacacatgcccaccgtgcccagcacctgaactcctggggggaccgtcagtcttcctcttccccccaaaacccaaggacaccctcatgatctcccggacccctgaggtcacatgcgtggtggtggacgtgagccacgaagaccctgaggtcaagttcaactggtacgtggacggcgtggaggtgcataatgccaagacaaagccgcgggaggagcagtacgccagcacgtaccgtgtggtcagcgtcctcaccgtcctgcaccaggactggctgaatggcaaggagtacaagtgcaaggtctccaacaaagccctcccagcccccatagagaaaaccatctccaaagccaaagggcagccccgagaaccacaggtgtacaccctgcccccatcccgggaggagatgaccaagaaccaggtcagcctgacctgcctggtcaaaggcttctatcccagcgacatcgccgtggagtgggagagcaatgggcagccggagaacaactacaagaccacgcctcccgtgctggactccgacggctccttcttcctctacagcaagctcaccgtggacaagagcaggtggcagcaggggaacgtcttctcatgctccgtgatgcatgaggctctgcacaaccactacacgcagaagagcctctccctgtctccgggtaaa

SEQ ID NO: 19 - DNA, 642 bp, synthetic construct
  source 1..642: mol_type = other DNA
gacatccagatgacccagagccccagcagcctgagcgccagcgtgggcgaccgcgtgaccatcacctgccgcgccagcgagagcgtggacgacctgctgcactggtaccagcagaagcccggcaaggcccccaagctgctgatcaagtacgccagccagagcatcagcggcgtgcccagccgcttcagcggcagcggcagcggcaccgacttcaccctgaccatcagcagcctgcagcccgaggacttcgccacctactactgccagcagggcaacagcctgcccaacaccttcggccagggcaccaaggtggagatcaagcgcacagtggcagcccccagcgtcttcatttttcccccttccgatgaacagctgaagtccggcactgcttctgtggtctgtctgctgaacaatttctatcccagagaggccaaggtgcagtggaaagtggacaacgctctgcagtccggcaacagccaggagagtgtgaccgaacaggatagtaaggacagcacatattctctgtctagtaccctgacactgagtaaggcagattacgagaagcacaaagtgtatgcctgcgaagtcactcatcagggactgtcaagccccgtgaccaagagcttcaaccggggcgagtgt

SEQ ID NO: 20 - DNA, 879 bp, synthetic construct
  source 1..879: mol_type = other DNA
gacatccagatgacccagagccccagcagcctgagcgccagcgtgggcgaccgcgtgaccatcacctgccgcgccagcgagagcggcggaagcggagcaaagctcgccgcactgaaagccaagctggccgctctgaagggaggtggcgggagcgccgctgcaatctcctgcgtcggcagccccgaatgtcctcccaagtgccgggctcagggatgcaagaacggcaagtgtatgaaccggaagtgcaagtgctactattgcggcggaggtgggagtgaactggccgcactggaagctgagctggctgccctcgaagctggaggctctggactgctgcactggtaccagcagaagcccggcaaggcccccaagctgctgatcaagtacgccagccagagcatcagcggcgtgcccagccgcttcagcggcagcggcagcggcaccgacttcaccctgaccatcagcagcctgcagcccgaggacttcgccacctactactgccagcagggcaacagcctgcccaacaccttcggccagggcaccaaggtggagatcaagcgcacagtggcagcccccagcgtcttcatttttcccccttccgatgaacagctgaagtccggcactgcttctgtggtctgtctgctgaacaatttctatcccagagaggccaaggtgcagtggaaagtggacaacgctctgcagtccggcaacagccaggagagtgtgaccgaacaggatagtaaggacagcacatattctctgtctagtaccctgacactgagtaaggcagattacgagaagcacaaagtgtatgcctgcgaagtcactcatcagggactgtcaagccccgtgaccaagagcttcaaccggggcgagtgt

SEQ ID NO: 21 - DNA, 879 bp, synthetic construct
  source 1..879: mol_type = other DNA
gacatccagatgacccagagccccagcagcctgagcgccagcgtgggcgaccgcgtgaccatcacctgccgcgccagcgagagcgtggacgacctgctgcactggtaccagcagaagcccggcaaggcccccaagctgctgatcaagtacgccagccagagcatcagcggcggaagcggagcaaagctcgccgcactgaaagccaagctggccgctctgaagggaggtggcgggagcgccgctgcaatctcctgcgtcggcagccccgaatgtcctcccaagtgccgggctcagggatgcaagaacggcaagtgtatgaaccggaagtgcaagtgctactattgcggcggaggtgggagtgaactggccgcactggaagctgagctggctgccctcgaagctggaggctctggaagccgcttcagcggcagcggcagcggcaccgacttcaccctgaccatcagcagcctgcagcccgaggacttcgccacctactactgccagcagggcaacagcctgcccaacaccttcggccagggcaccaaggtggagatcaagcgcacagtggcagcccccagcgtcttcatttttcccccttccgatgaacagctgaagtccggcactgcttctgtggtctgtctgctgaacaatttctatcccagagaggccaaggtgcagtggaaagtggacaacgctctgcagtccggcaacagccaggagagtgtgaccgaacaggatagtaaggacagcacatattctctgtctagtaccctgacactgagtaaggcagattacgagaagcacaaagtgtatgcctgcgaagtcactcatcagggactgtcaagccccgtgaccaagagcttcaaccggggcgagtgt

SEQ ID NO: 22 - DNA, 876 bp, synthetic construct
  source 1..876: mol_type = other DNA
gacatccagatgacccagagccccagcagcctgagcgccagcgtgggcgaccgcgtgaccatcacctgccgcgccagcgagagcgtggacgacctgctgcactggtaccagcagaagcccggcaaggcccccaagctgctgatcaagtacgccagccagagcatcagcggcgtgcccagccgcttcagcggcagcggcagcggcaccgacttcaccctgaccatcagcagcctgcagcccgaggacttcgccacctactactgccagcagggcggcggaagcggagcaaagctcgccgcactgaaagccaagctggccgctctgaagggaggtggcgggagcgccgctgcaatctcctgcgtcggcagccccgaatgtcctcccaagtgccgggctcagggatgcaagaacggcaagtgtatgaaccggaagtgcaagtgctactattgcggcggaggtgggagtgaactggccgcactggaagctgagctggctgccctcgaagctggaggctctggaaacaccttcggccagggcaccaaggtggagatcaagcgcacagtggcagcccccagcgtcttcatttttcccccttccgatgaacagctgaagtccggcactgcttctgtggtctgtctgctgaacaatttctatcccagagaggccaaggtgcagtggaaagtggacaacgctctgcagtccggcaacagccaggagagtgtgaccgaacaggatagtaaggacagcacatattctctgtctagtaccctgacactgagtaaggcagattacgagaagcacaaagtgtatgcctgcgaagtcactcatcagggactgtcaagccccgtgaccaagagcttcaaccggggcgagtgt

SEQ ID NO: 23 - DNA, 1569 bp, synthetic construct
  source 1..1569: mol_type = other DNA
gaggtgcagctggtggagagcggcggcggcctggtgcagcccggcggcagcctgcgcctgagctgcgccgccagcggcggcggaagcggagcaaagctcgccgcactgaaagccaagctggccgctctgaagggaggtggcgggagcgccgctgcaatctcctgcgtcggcagccccgaatgtcctcccaagtgccgggctcagggatgcaagaacggcaagtgtatgaaccggaagtgcaagtgctactattgcggcggaggtgggagtgaactggccgcactggaagctgagctggctgccctcgaagctggaggctctggatactggggctgggtgcgccaggcccccggcaagggcctggagtgggtgggctacatcagctacagcggcagcaccagctacaaccccagcctgaagagccgcttcaccatcagccgcgacaccagcaagaacaccttctacctgcagatgaacagcctgcgcgccgaggacaccgccgtgtactactgcgcccgcaccggcagcagcggctacttcgacttctggggccagggcaccctggtgaccgtgagcagcgcctccaccaagggcccatcggtcttccccctggcaccctcctccaagagcacctctgggggcacagcggccctgggctgcctggtcaaggactacttccccgaaccggtgacggtgtcgtggaactcaggcgccctgaccagcggcgtgcacaccttcccggctgtcctacagtcctcaggactctactccctcagcagcgtggtgactgtgccctctagcagcttgggcacccagacctacatctgcaacgtgaatcacaagcccagcaacaccaaggtggacaagaaagttgaacccaaatcttgcgacaaaactcacacatgcccaccgtgcccagcacctgaactcctggggggaccgtcagtcttcctcttccccccaaaacccaaggacaccctcatgatctcccggacccctgaggtcacatgcgtggtggtggacgtgagccacgaagaccctgaggtcaagttcaactggtacgtggacggcgtggaggtgcataatgccaagacaaagccgcgggaggagcagtacgccagcacgtaccgtgtggtcagcgtcctcaccgtcctgcaccaggactggctgaatggcaaggagtacaagtgcaaggtctccaacaaagccctcccagcccccatagagaaaaccatctccaaagccaaagggcagccccgagaaccacaggtgtacaccctgcccccatcccgggaggagatgaccaagaaccaggtcagcctgacctgcctggtcaaaggcttctatcccagcgacatcgccgtggagtgggagagcaatgggcagccggagaacaactacaagaccacgcctcccgtgctggactccgacggctccttcttcctctacagcaagctcaccgtggacaagagcaggtggcagcaggggaacgtcttctcatgctccgtgatgcatgaggctctgcacaaccactacacgcagaagagcctctccctgtctccgggtaaa

SEQ ID NO: 24 - DNA, 1575 bp, synthetic construct
  source 1..1575: mol_type = other DNA
gaggtgcagctggtggagagcggcggcggcctggtgcagcccggcggcagcctgcgcctgagctgcgccgccagcggcttcttcatcaccaacaactactggggctgggtgcgccaggcccccggcaagggcctggagtgggtgggctacatcagctacagcggcagcaccagctacaacggcggaagcggagcaaagctcgccgcactgaaagccaagctggccgctctgaagggaggtggcgggagcgccgctgcaatctcctgcgtcggcagccccgaatgtcctcccaagtgccgggctcagggatgcaagaacggcaagtgtatgaaccggaagtgcaagtgctactattgcggcggaggtgggagtgaactggccgcactggaagctgagctggctgccctcgaagctggaggctctggaagccgcttcaccatcagccgcgacaccagcaagaacaccttctacctgcagatgaacagcctgcgcgccgaggacaccgccgtgtactactgcgcccgcaccggcagcagcggctacttcgacttctggggccagggcaccctggtgaccgtgagcagcgcctccaccaagggcccatcggtcttccccctggcaccctcctccaagagcacctctgggggcacagcggccctgggctgcctggtcaaggactacttccccgaaccggtgacggtgtcgtggaactcaggcgccctgaccagcggcgtgcacaccttcccggctgtcctacagtcctcaggactctactccctcagcagcgtggtgactgtgccctctagcagcttgggcacccagacctacatctgcaacgtgaatcacaagcccagcaacaccaaggtggacaagaaagttgaacccaaatcttgcgacaaaactcacacatgcccaccgtgcccagcacctgaactcctggggggaccgtcagtcttcctcttccccccaaaacccaaggacaccctcatgatctcccggacccctgaggtcacatgcgtggtggtggacgtgagccacgaagaccctgaggtcaagttcaactggtacgtggacggcgtggaggtgcataatgccaagacaaagccgcgggaggagcagtacgccagcacgtaccgtgtggtcagcgtcctcaccgtcctgcaccaggactggctgaatggcaaggagtacaagtgcaaggtctccaacaaagccctcccagcccccatagagaaaaccatctccaaagccaaagggcagccccgagaaccacaggtgtacaccctgcccccatcccgggaggagatgaccaagaaccaggtcagcctgacctgcctggtcaaaggcttctatcccagcgacatcgccgtggagtgggagagcaatgggcagccggagaacaactacaagaccacgcctcccgtgctggactccgacggctccttcttcctctacagcaagctcaccgtggacaagagcaggtggcagcaggggaacgtcttctcatgctccgtgatgcatgaggctctgcacaaccactacacgcagaagagcctctccctgtctccgggtaaa

SEQ ID NO: 25 - DNA, 1575 bp, synthetic construct
  source 1..1575: mol_type = other DNA
gaggtgcagctggtggagagcggcggcggcctggtgcagcccggcggcagcctgcgcctgagctgcgccgccagcggcttcttcatcaccaacaactactggggctgggtgcgccaggcccccggcaagggcctggagtgggtgggctacatcagctacagcggcagcaccagctacaaccccagcctgaagagccgcttcaccatcagccgcgacaccagcaagaacaccttctacctgcagatgaacagcctgcgcgccgaggacaccgccgtgtactactgcgcccgcggcggaagcggagcaaagctcgccgcactgaaagccaagctggccgctctgaagggaggtggcgggagcgccgctgcaatctcctgcgtcggcagccccgaatgtcctcccaagtgccgggctcagggatgcaagaacggcaagtgtatgaaccggaagtgcaagtgctactattgcggcggaggtgggagtgaactggccgcactggaagctgagctggctgccctcgaagctggaggctctggaggctacttcgacttctggggccagggcaccctggtgaccgtgagcagcgcctccaccaagggcccatcggtcttccccctggcaccctcctccaagagcacctctgggggcacagcggccctgggctgcctggtcaaggactacttccccgaaccggtgacggtgtcgtggaactcaggcgccctgaccagcggcgtgcacaccttcccggctgtcctacagtcctcaggactctactccctcagcagcgtggtgactgtgccctctagcagcttgggcacccagacctacatctgcaacgtgaatcacaagcccagcaacaccaaggtggacaagaaagttgaacccaaatcttgcgacaaaactcacacatgcccaccgtgcccagcacctgaactcctggggggaccgtcagtcttcctcttccccccaaaacccaaggacaccctcatgatctcccggacccctgaggtcacatgcgtggtggtggacgtgagccacgaagaccctgaggtcaagttcaactggtacgtggacggcgtggaggtgcataatgccaagacaaagccgcgggaggagcagtacgccagcacgtaccgtgtggtcagcgtcctcaccgtcctgcaccaggactggctgaatggcaaggagtacaagtgcaaggtctccaacaaagccctcccagcccccatagagaaaaccatctccaaagccaaagggcagccccgagaaccacaggtgtacaccctgcccccatcccgggaggagatgaccaagaaccaggtcagcctgacctgcctggtcaaaggcttctatcccagcgacatcgccgtggagtgggagagcaatgggcagccggagaacaactacaagaccacgcctcccgtgctggactccgacggctccttcttcctctacagcaagctcaccgtggacaagagcaggtggcagcaggggaacgtcttctcatgctccgtgatgcatgaggctctgcacaaccactacacgcagaagagcctctccctgtctccgggtaaa

SEQ ID NO: 26 - DNA, 108 bp, synthetic construct
  source 1..108: mol_type = other DNA
gccgctgcaatctcctgcgtcggcagccccgaatgtcctcccaagtgccgggctcagggatgcaagaacggcaagtgtatgaaccggaagtgcaagtgctactattgc